European Patent Application EP 4 339 207 A1, published March 20, 2024. Title: ANTIGEN BINDING MOLECULE SPECIFICALLY BINDING TO RANKL AND NGF, AND MEDICAL USE THEREOF. Applicant: JIANGSU HENGRUI PHARMACEUTICALS CO., LTD. SHANGHAI HENGRUI PHARMACEUTICAL CO., LTD. Application PCT/CN2022/092333. The sequence listing filed with the application follows.

SEQUENCE LISTING (111 sequences)

SEQ ID NO: 1 - protein, 5 aa, Artificial sequence
  1-22H HCDR1
DYAMS

SEQ ID NO: 2 - protein, 17 aa, Artificial sequence
  1-22H HCDR2
GISASGSSTYYADSVKG

SEQ ID NO: 3 - protein, 13 aa, Artificial sequence
  1-22H HCDR3
DPGTTVIMSWFDP

SEQ ID NO: 4 - protein, 12 aa, Artificial sequence
  1-22H LCDR1
RASQSVRGRYLA

SEQ ID NO: 5 - protein, 7 aa, Artificial sequence
  1-22H LCDR2
GASSRAT

SEQ ID NO: 6 - protein, 9 aa, Artificial sequence
  1-22H LCDR3
QQYGSSPRT

SEQ ID NO: 7 - protein, 5 aa, Artificial sequence
  5-16H HCDR1
SYAMS

SEQ ID NO: 8 - protein, 17 aa, Artificial sequence
  5-16H HCDR2
GITGSGGSTYYADSVKG

SEQ ID NO: 9 - protein, 13 aa, Artificial sequence
  5-16H HCDR3
DPASIVIMSWFDP

SEQ ID NO: 10 - protein, 13 aa, Artificial sequence
  5-51H HCDR3
DPCFSYIMSWFDP

SEQ ID NO: 11 - protein, 13 aa, Artificial sequence
  5-53H HCDR3
DPCFTYIMSWFDP

SEQ ID NO: 12 - protein, 13 aa, Artificial sequence
  5-58H HCDR3
DPGFTYIMSWFDP

SEQ ID NO: 13 - protein, 5 aa, Artificial sequence
  D35H HCDR1
AYPMS

SEQ ID NO: 14 - protein, 13 aa, Artificial sequence
  D75H HCDR3
DPGTTSIMSWFDP

SEQ ID NO: 15 - protein, 13 aa, Artificial sequence
  D80H HCDR3
DPGSTIIMSWFDP

SEQ ID NO: 16 - protein, 7 aa, Artificial sequence
  2-52L LCDR2
QGSSRAT

SEQ ID NO: 17 - protein, 12 aa, Artificial sequence
  2-72L LCDR1
RASQSLGARGLA

SEQ ID NO: 18 - protein, 7 aa, Artificial sequence
  2-72L LCDR2
GTSSRAT

SEQ ID NO: 19 - protein, 12 aa, Artificial sequence
  2-76L LCDR1
RASQAIPYNQLA

SEQ ID NO: 20 - protein, 7 aa, Artificial sequence
  2-76L LCDR2
GVSSRAT

SEQ ID NO: 21 - protein, 7 aa, Artificial sequence
  2-79L LCDR2
GSSSRAT

SEQ ID NO: 22 - protein, 12 aa, Artificial sequence
  2-87L LCDR1
RASQYLPFHRLA

SEQ ID NO: 23 - protein, 7 aa, Artificial sequence
  2-87L LCDR2
DTSSRAT

SEQ ID NO: 24 - protein, 12 aa, Artificial sequence
  3-20L LCDR1
RASQAIRGPNLA

SEQ ID NO: 25 - protein, 7 aa, Artificial sequence
  3-20L LCDR2
DTSSRAT

SEQ ID NO: 26 - protein, 12 aa, Artificial sequence
  3-37L LCDR1
RASQAIRGRKLA

SEQ ID NO: 27 - protein, 7 aa, Artificial sequence
  3-37L LCDR2
DTSSRAT

SEQ ID NO: 28 - protein, 12 aa, Artificial sequence
  3-83L LCDR1
RASQALGVRGLA

SEQ ID NO: 29 - protein, 12 aa, Artificial sequence
  3-85L LCDR1
RASQSIPGPRLA

SEQ ID NO: 30 - protein, 9 aa, Artificial sequence
  4-64L LCDR3
QQYGSSPRI

SEQ ID NO: 31 - protein, 122 aa, Artificial sequence
  1-22H heavy chain variable region
EVQLLESGGGLVQPGGSLRLSCAASGFTFADYAMSWVRQAPGKGLEWVSGISASGSSTYYADSVKGRFTISRDNSKNTLYLQMNSLRAEDTAVYYCAKDPGTTVIMSWFDPWGQGTLVTVSS

SEQ ID NO: 32 - protein, 122 aa, Artificial sequence
  5-16H heavy chain variable region
EVQLLESGGGLVQPGGSLRLSCAASGFTFSSYAMSWVRQAPGKGLEWVSGITGSGGSTYYADSVKGRFTISRDNSKNTLYLQMNSLRAEDTAVYYCAKDPASIVIMSWFDPWGQGTLVTVSS

SEQ ID NO: 33 - protein, 122 aa, Artificial sequence
  5-51H heavy chain variable region
EVQLLESGGGLVQPGGSLRLSCAASGFTFSSYAMSWVRQAPGKGLEWVSGITGSGGSTYYADSVKGRFTISRDNSKNTLYLQMNSLRAEDTAVYYCAKDPCFSYIMSWFDPWGQGTLVTVSS

SEQ ID NO: 34 - protein, 122 aa, Artificial sequence
  5-53H heavy chain variable region
EVQLLESGGGLVQPGGSLRLSCAASGFTFSSYAMSWVRQAPGKGLEWVSGITGSGGSTYYADSVKGRFTISRDNSKNTLYLQMNSLRAEDTAVYYCAQDPCFTYIMSWFDPWGQGTLVTVSS

SEQ ID NO: 35 - protein, 122 aa, Artificial sequence
  5-58H heavy chain variable region
EVQLLESGGGLVQPGGSLRLSCAASGFTFSSYAMSWVRQAPGKGLEWVSGITGSGGSTYYADSVKGRFTISRDNSKNTLYLQMNSLRAEDTAVYYCVQDPGFTYIMSWFDPWGQGTLVTVSS

SEQ ID NO: 36 - protein, 122 aa, Artificial sequence
  D35H heavy chain variable region
EVQLLESGGGLVQPGGSLRLSCAASGFTFSAYPMSWVRQAPGKGLEWVSGITGSGGSTYYADSVKGRFTISRDNSKNTLYLQMNSLRAEDTAVYYCAKDPGTTVIMSWFDPWGQGTLVTVSS

SEQ ID NO: 37 - protein, 122 aa, Artificial sequence
  D75H heavy chain variable region
EVQLLESGGGLVQPGGSLRLSCAASGFTFSSYAMSWVRQAPGKGLEWVSGITGSGGSTYYADSVKGRFTISRDNSKNTLYLQMNSLRAEDTAVYYCVKDPGTTSIMSWFDPWGQGTLVTVSS

SEQ ID NO: 38 - protein, 122 aa, Artificial sequence
  D80H heavy chain variable region
EVQLLESGGGLVQPGGSLRLSCAASGFTFSSYAMSWVRQAPGKGLEWVSGITGSGGSTYYADSVKGRFTISRDNSKNTLYLQMNSLRAEDTAVYYCVKDPGSTIIMSWFDPWGQGTLVTVSS

SEQ ID NO: 39 - protein, 122 aa, Artificial sequence
  2-52L heavy chain variable region
EVQLLESGGGLVQPGGSLRLSCAASGFTFSSYAMSWVRQAPGKGLEWVSGITGSGGSTYYADSVKGRFTISRDNSKNTLYLQMNSLRAEDTAVYYCAKDPGTTVIMSWFDPWGQGTLVTVSS

SEQ ID NO: 40 - protein, 108 aa, Artificial sequence
  Light chain variable region
EIVLTQSPGTLSLSPGERATLSCRASQSVRGRYLAWYQQKPGQAPRLLIYGASSRATGIPDRFSGSGSGTDFTLTISRLEPEDFAVFYCQQYGSSPRTFGQGTKVEIK

SEQ ID NO: 41 - protein, 108 aa, Artificial sequence
  2-52L light chain variable region
EIVLTQSPGTLSLSPGERATLSCRASQSVRGRYLAWYQQKPGQAPRLLIYQGSSRATGIPDRFSGSGSGTDFTLTISRLEPEDFAVFYCQQYGSSPRTFGQGTKVEIK

SEQ ID NO: 42 - protein, 108 aa, Artificial sequence
  2-72L light chain variable region
EIVLTQSPGTLSLSPGERATLSCRASQSLGARGLAWYQQKPGQAPRLLIYGTSSRATGIPDRFSGSGSGTDFTLTISRLEPEDFAVFYCQQYGSSPRTFGQGTKVEIK

SEQ ID NO: 43 - protein, 108 aa, Artificial sequence
  2-76L light chain variable region
EIVLTQSPGTLSLSPGERATLSCRASQAIPYNQLAWYQQKPGQAPRLLIYGVSSRATGIPDRFSGSGSGTDFTLTISRLEPEDFAVFYCQQYGSSPRTFGQGTKVEIK

SEQ ID NO: 44 - protein, 108 aa, Artificial sequence
  2-79L light chain variable region
EIVLTQSPGTLSLSPGERATLSCRASQSVRGRYLAWYQQKPGQAPRLLIYGSSSRATGIPDRFSGSGSGTDFTLTISRLEPEDFAVFYCQQYGSSPRTFGQGTKVEIK

SEQ ID NO: 45 - protein, 108 aa, Artificial sequence
  2-87L light chain variable region
EIVLTQSPGTLSLSPGERATLSCRASQYLPFHRLAWYQQKPGQAPRLLIYDTSSRATGIPDRFSGSGSGTDFTLTISRLEPEDFAVFYCQQYGSSPRTFGQGTKVEIK

SEQ ID NO: 46 - protein, 108 aa, Artificial sequence
  3-20L light chain variable region
EIVLTQSPGTLSLSPGERATLSCRASQAIRGPNLAWYQQKPGQAPRLLIYDTSSRATGIPDRFSGSGSGTDFTLTISRLEPEDFAVFYCQQYGSSPRTFGQGTKVEIK

SEQ ID NO: 47 - protein, 108 aa, Artificial sequence
  3-37L light chain variable region
EIVLTQSPGTLSLSPGERATLSCRASQAIRGRKLAWYQQKPGQAPRLLIYDTSSRATGIPDRFSGSGSGTDFTLTISRLEPEDFAVFYCQQYGSSPRTFGQGTKVEIK

SEQ ID NO: 48 - protein, 108 aa, Artificial sequence
  3-83L light chain variable region
EIVLTQSPGTLSLSPGERATLSCRASQALGVRGLAWYQQKPGQAPRLLIYGASSRATGIPDRFSGSGSGTDFTLTISRLEPEDFAVFYCQQYGSSPRTFGQGTKVEIK

SEQ ID NO: 49 - protein, 108 aa, Artificial sequence
  3-85L light chain variable region
EIVLTQSPGTLSLSPGERATLSCRASQSIPGPRLAWYQQKPGQAPRLLIYGASSRATGIPDRFSGSGSGTDFTLTISRLEPEDFAVFYCQQYGSSPRTFGQGTKVEIK

SEQ ID NO: 50 - protein, 108 aa, Artificial sequence
  4-64L light chain variable region
EIVLTQSPGTLSLSPGERATLSCRASQSVRGRYLAWYQQKPGQAPRLLIYGASSRATGIPDRFSGSGSGTDFTLTISRLEPEDFAVFYCQQYGSSPRIFGQGTKVEIK

SEQ ID NO: 51 - protein, 327 aa, homo sapiens
ASTKGPSVFPLAPCSRSTSESTAALGCLVKDYFPEPVTVSWNSGALTSGVHTFPAVLQSSGLYSLSSVVTVPSSSLGTKTYTCNVDHKPSNTKVDKRVESKYGPPCPPCPAPEFLGGPSVFLFPPKPKDTLMISRTPEVTCVVVDVSQEDPEVQFNWYVDGVEVHNAKTKPREEQFNSTYRVVSVLTVLHQDWLNGKEYKCKVSNKGLPSSIEKTISKAKGQPREPQVYTLPPSQEEMTKNQVSLTCLVKGFYPSDIAVEWESNGQPENNYKTTPPVLDSDGSFFLYSRLTVDKSRWQEGNVFSCSVMHEALHNHYTQKSLSLSLGK

SEQ ID NO: 52 - protein, 107 aa, homo sapiens [sequence omitted]

SEQ ID NO: 53 - protein, 449 aa, Artificial sequence
  D35H heavy chain
EVQLLESGGGLVQPGGSLRLSCAASGFTFSAYPMSWVRQAPGKGLEWVSGITGSGGSTYYADSVKGRFTISRDNSKNTLYLQMNSLRAEDTAVYYCAKDPGTTVIMSWFDPWGQGTLVTVSSASTKGPSVFPLAPCSRSTSESTAALGCLVKDYFPEPVTVSWNSGALTSGVHTFPAVLQSSGLYSLSSVVTVPSSSLGTKTYTCNVDHKPSNTKVDKRVESKYGPPCPPCPAPEFLGGPSVFLFPPKPKDTLMISRTPEVTCVVVDVSQEDPEVQFNWYVDGVEVHNAKTKPREEQFNSTYRVVSVLTVLHQDWLNGKEYKCKVSNKGLPSSIEKTISKAKGQPREPQVYTLPPSQEEMTKNQVSLTCLVKGFYPSDIAVEWESNGQPENNYKTTPPVLDSDGSFFLYSRLTVDKSRWQEGNVFSCSVMHEALHNHYTQKSLSLSLGK

SEQ ID NO: 54 - protein, 215 aa, Artificial sequence
  D35H light chain
EIVLTQSPGTLSLSPGERATLSCRASQSVRGRYLAWYQQKPGQAPRLLIYGASSRATGIPDRFSGSGSGTDFTLTISRLEPEDFAVFYCQQYGSSPRTFGQGTKVEIKRTVAAPSVFIFPPSDEQLKSGTASVVCLLNNFYPREAKVQWKVDNALQSGNSQESVTEQDSKDSTYSLSSTLTLSKADYEKHKVYACEVTHQGLSSPVTKSFNRGEC

SEQ ID NO: 55 - protein, 509 aa, Artificial sequence
  D75H heavy chain
EIVLTQSPGTLSLSPGERATLSCRASQSVRGRYLAWYQQKPGQAPRLLIYGASSRATGIPEVQLLESGGGLVQPGGSLRLSCAASGFTFSSYAMSWVRQAPGKGLEWVSGITGSGGSTYYADSVKGRFTISRDNSKNTLYLQMNSLRAEDTAVYYCVKDPGTTSIMSWFDPWGQGTLVTVSSASTKGPSVFPLAPCSRSTSESTAALGCLVKDYFPEPVTVSWNSGALTSGVHTFPAVLQSSGLYSLSSVVTVPSSSLGTKTYTCNVDHKPSNTKVDKRVESKYGPPCPPCPAPEFLGGPSVFLFPPKPKDTLMISRTPEVTCVVVDVSQEDPEVQFNWYVDGVEVHNAKTKPREEQFNSTYRVVSVLTVLHQDWLNGKEYKCKVSNKGLPSSIEKTISKAKGQPREPQVYTLPPSQEEMTKNQVSLTCLVKGFYPSDIAVEWESNGQPENNYKTTPPVLDSDGSFFLYSRLTVDKSRWQEGNVFSCSVMHEALHNHYTQKSLSLSLGK

SEQ ID NO: 56 - protein, 449 aa, Artificial sequence
  D80H heavy chain
EVQLLESGGGLVQPGGSLRLSCAASGFTFSSYAMSWVRQAPGKGLEWVSGITGSGGSTYYADSVKGRFTISRDNSKNTLYLQMNSLRAEDTAVYYCVKDPGSTIIMSWFDPWGQGTLVTVSSASTKGPSVFPLAPCSRSTSESTAALGCLVKDYFPEPVTVSWNSGALTSGVHTFPAVLQSSGLYSLSSVVTVPSSSLGTKTYTCNVDHKPSNTKVDKRVESKYGPPCPPCPAPEFLGGPSVFLFPPKPKDTLMISRTPEVTCVVVDVSQEDPEVQFNWYVDGVEVHNAKTKPREEQFNSTYRVVSVLTVLHQDWLNGKEYKCKVSNKGLPSSIEKTISKAKGQPREPQVYTLPPSQEEMTKNQVSLTCLVKGFYPSDIAVEWESNGQPENNYKTTPPVLDSDGSFFLYSRLTVDKSRWQEGNVFSCSVMHEALHNHYTQKSLSLSLGK

SEQ ID NO: 57 - protein, 448 aa, Artificial sequence
  Denosumab heavy chain
EVQLLESGGGLVQPGGSLRLSCAASGFTFSSYAMSWVRQAPGKGLEWVSGITGSGGSTYYADSVKGRFTISRDNSKNTLYLQMNSLRAEDTAVYYCAKDPGTTVIMSWFDPWGQGTLVTVSSASTKGPSVFPLAPCSRSTSESTAALGCLVKDYFPEPVTVSWNSGALTSGVHTFPAVLQSSGLYSLSSVVTVPSSNFGTQTYTCNVDHKPSNTKVDKTVERKCCVECPPCPAPPVAGPSVFLFPPKPKDTLMISRTPEVTCVVVDVSHEDPEVQFNWYVDGVEVHNAKTKPREEQFNSTFRVVSVLTVVHQDWLNGKEYKCKVSNKGLPAPIEKTISKTKGQPREPQVYTLPPSREEMTKNQVSLTCLVKGFYPSDIAVEWESNGQPENNYKTTPPMLDSDGSFFLYSKLTVDKSRWQQGNVFSCSVMHEALHNHYTQKSLSLSPGK

SEQ ID NO: 58 - protein, 5 aa, Artificial sequence
  Tanezumab HCDR1
GYDLN

SEQ ID NO: 59 - protein, 16 aa, Artificial sequence
  Tanezumab HCDR2
IIWGDGTTDYNSAVKS

SEQ ID NO: 60 - protein, 13 aa, Artificial sequence
  Tanezumab HCDR3
GGYWYATSYYFDY

SEQ ID NO: 61 - protein, 11 aa, Artificial sequence
  Tanezumab LCDR1
RASQSISNNLN

SEQ ID NO: 62 - protein, 7 aa, Artificial sequence
  Tanezumab LCDR2
YTSRFHS

SEQ ID NO: 63 - protein, 13 aa, Artificial sequence
  Tanezumab LCDR3
GGYWYATSYYFDY

SEQ ID NO: 64 - protein, 121 aa, Artificial sequence [sequence omitted]

SEQ ID NO: 65 - protein, 107 aa, Artificial sequence [sequence omitted]

SEQ ID NO: 66 - protein, 326 aa, Artificial sequence
  Heavy chain constant region
ASTKGPSVFPLAPCSRSTSESTAALGCLVKDYFPEPVTVSWNSGALTSGVHTFPAVLQSSGLYSLSSVVTVPSSNFGTQTYTCNVDHKPSNTKVDKTVERKCCVECPPCPAPPVAGPSVFLFPPKPKDTLMISRTPEVTCVVVDVSHEDPEVQFNWYVDGVEVHNAKTKPREEQFNSTFRVVSVLTVVHQDWLNGKEYKCKVSNKGLPSSIEKTISKTKGQPREPQVYTLPPSREEMTKNQVSLTCLVKGFYPSDIAVEWESNGQPENNYKTTPPMLDSDGSFFLYSKLTVDKSRWQQGNVFSCSVMHEALHNHYTQKSLSLSPGK

SEQ ID NO: 67 - protein, 448 aa, Artificial sequence
  N-mAb heavy chain
QVQLQESGPGLVKPSETLSLTCTVSGFSLIGYDLNWIRQPPGKGLEWIGIIWGDGTTDYNSAVKSRVTISKDTSKNQFSLKLSSVTAADTAVYYCARGGYWYATSYYFDYWGQGTLVTVSSASTKGPSVFPLAPCSRSTSESTAALGCLVKDYFPEPVTVSWNSGALTSGVHTFPAVLQSSGLYSLSSVVTVPSSSLGTKTYTCNVDHKPSNTKVDKRVESKYGPPCPPCPAPEFLGGPSVFLFPPKPKDTLMISRTPEVTCVVVDVSQEDPEVQFNWYVDGVEVHNAKTKPREEQFNSTYRVVSVLTVLHQDWLNGKEYKCKVSNKGLPSSIEKTISKAKGQPREPQVYTLPPSQEEMTKNQVSLTCLVKGFYPSDIAVEWESNGQPENNYKTTPPVLDSDGSFFLYSRLTVDKSRWQEGNVFSCSVMHEALHNHYTQKSLSLSLGK

SEQ ID NO: 68 - protein, 214 aa, Artificial sequence
  N-mAb light chain
DIQMTQSPSSLSASVGDRVTITCRASQSISNNLNWYQQKPGKAPKLLIYYTSRFHSGVPSRFSGSGSGTDFTFTISSLQPEDIATYYCQQEHTLPYTFGQGTKLEIKRTVAAPSVFIFPPSDEQLKSGTASVVCLLNNFYPREAKVQWKVDNALQSGNSQESVTEQDSKDSTYSLSSTLTLSKADYEKHKVYACEVTHQGLSSPVTKSFNRGEC

SEQ ID NO: 69 - protein, 447 aa, Artificial sequence
  Tanezumab heavy chain
QVQLQESGPGLVKPSETLSLTCTVSGFSLIGYDLNWIRQPPGKGLEWIGIIWGDGTTDYNSAVKSRVTISKDTSKNQFSLKLSSVTAADTAVYYCARGGYWYATSYYFDYWGQGTLVTVSSASTKGPSVFPLAPCSRSTSESTAALGCLVKDYFPEPVTVSWNSGALTSGVHTFPAVLQSSGLYSLSSVVTVPSSNFGTQTYTCNVDHKPSNTKVDKTVERKCCVECPPCPAPPVAGPSVFLFPPKPKDTLMISRTPEVTCVVVDVSHEDPEVQFNWYVDGVEVHNAKTKPREEQFNSTFRVVSVLTVVHQDWLNGKEYKCKVSNKGLPSSIEKTISKTKGQPREPQVYTLPPSREEMTKNQVSLTCLVKGFYPSDIAVEWESNGQPENNYKTTPPMLDSDGSFFLYSKLTVDKSRWQQGNVFSCSVMHEALHNHYTQKSLSLSPGK

SEQ ID NO: 70 - protein, 6 aa, Artificial sequence
  Linker
ASTKGP

SEQ ID NO: 71 - protein, 6 aa, Artificial sequence
  Linker
TVAAPS

SEQ ID NO: 72 - protein, 13 aa, Artificial sequence
  Linker
ASTKGPSVFPLAP

SEQ ID NO: 73 - protein, 12 aa, Artificial sequence
  Linker
TVAAPSVFIFPP

SEQ ID NO: 74 - protein, 16 aa, Artificial sequence
  Linker
AKTTPKLEEGEFSEAR

SEQ ID NO: 75 - protein, 17 aa, Artificial sequence
  Linker
AKTTPKLEEGEFSEARV

SEQ ID NO: 76 - protein, 9 aa, Artificial sequence
  Linker
AKTTPKLGG

SEQ ID NO: 77 - protein, 10 aa, Artificial sequence
  Linker
SAKTTPKLGG

SEQ ID NO: 78 - protein, 6 aa, Artificial sequence
  Linker
SAKTTP

SEQ ID NO: 79 - protein, 6 aa, Artificial sequence
  Linker
RADAAP

SEQ ID NO: 80 - protein, 9 aa, Artificial sequence
  Linker
RADAAPTVS

SEQ ID NO: 81 - protein, 12 aa, Artificial sequence
  Linker
RADAAAAGGPGS

SEQ ID NO: 82 - protein, 18 aa, Artificial sequence
  Linker
SAKTTPKLEEGEFSEARV

SEQ ID NO: 83 - protein, 5 aa, Artificial sequence
  Linker
ADAAP

SEQ ID NO: 84 - protein, 12 aa, Artificial sequence
  Linker
ADAAPTVSIFPP

SEQ ID NO: 85 - protein, 5 aa, Artificial sequence
  Linker
TVAAP

SEQ ID NO: 86 - protein, 12 aa, Artificial sequence
  Linker
TVAAPSVFIFPP

SEQ ID NO: 87 - protein, 6 aa, Artificial sequence
  Linker
QPKAAP

SEQ ID NO: 88 - protein, 13 aa, Artificial sequence
  Linker
QPKAAPSVTLFPP

SEQ ID NO: 89 - protein, 6 aa, Artificial sequence
  Linker
AKTTPP

SEQ ID NO: 90 - protein, 13 aa, Artificial sequence
  Linker
AKTTPPSVTPLAP

SEQ ID NO: 91 - protein, 6 aa, Artificial sequence
  Linker
AKTTAP

SEQ ID NO: 92 - protein, 13 aa, Artificial sequence
  Linker
AKTTAPSVYPLAP

SEQ ID NO: 93 - protein, 13 aa, Artificial sequence
  Linker
ASTKGPSVFPLAP

SEQ ID NO: 94 - protein, 15 aa, Artificial sequence
  Linker
GGGGSGGGGSGGGGS

SEQ ID NO: 95 - protein, 15 aa, Artificial sequence
  Linker
GENKVEYAPALMALS

SEQ ID NO: 96 - protein, 15 aa, Artificial sequence
  Linker
GPAKELTPLKEAKVS

SEQ ID NO: 97 - protein, 15 aa, Artificial sequence
  Linker
GHEAAAVMQVQYPAS

SEQ ID NO: 98 - protein, 576 aa, Artificial sequence
  First chain of bispecific antibody 1
EVQLLESGGGLVQPGGSLRLSCAASGFTFSSYAMSWVRQAPGKGLEWVSGITGSGGSTYYADSVKGRFTISRDNSKNTLYLQMNSLRAEDTAVYYCVKDPGTTSIMSWFDPWGQGTLVTVSSASTKGPQVQLQESGPGLVKPSETLSLTCTVSGFSLIGYDLNWIRQPPGKGLEWIGIIWGDGTTDYNSAVKSRVTISKDTSKNQFSLKLSSVTAADTAVYYCARGGYWYATSYYFDYWGQGTLVTVSSASTKGPSVFPLAPCSRSTSESTAALGCLVKDYFPEPVTVSWNSGALTSGVHTFPAVLQSSGLYSLSSVVTVPSSSLGTKTYTCNVDHKPSNTKVDKRVESKYGPPCPPCPAPEFLGGPSVFLFPPKPKDTLMISRTPEVTCVVVDVSQEDPEVQFNWYVDGVEVHNAKTKPREEQFNSTYRVVSVLTVLHQDWLNGKEYKCKVSNKGLPSSIEKTISKAKGQPREPQVYTLPPSQEEMTKNQVSLTCLVKGFYPSDIAVEWESNGQPENNYKTTPPVLDSDGSFFLYSRLTVDKSRWQEGNVFSCSVMHEALHNHYTQKSLSLSLGK

SEQ ID NO: 99 - protein, 327 aa, Artificial sequence
  Second chain of bispecific antibody 1
EIVLTQSPGTLSLSPGERATLSCRASQSVRGRYLAWYQQKPGQAPRLLIYGASSRATGIPDRFSGSGSGTDFTLTISRLEPEDFAVFYCQQYGSSPRTFGQGTKVEIKTVAAPDIQMTQSPSSLSASVGDRVTITCRASQSISNNLNWYQQKPGKAPKLLIYYTSRFHSGVPSRFSGSGSGTDFTFTISSLQPEDIATYYCQQEHTLPYTFGQGTKLEIKRTVAAPSVFIFPPSDEQLKSGTASVVCLLNNFYPREAKVQWKVDNALQSGNSQESVTEQDSKDSTYSLSSTLTLSKADYEKHKVYACEVTHQGLSSPVTKSFNRGEC

SEQ ID NO: 100 - protein, 576 aa, Artificial sequence
  First chain of bispecific antibody 2
EVQLLESGGGLVQPGGSLRLSCAASGFTFSAYPMSWVRQAPGKGLEWVSGITGSGGSTYYADSVKGRFTISRDNSKNTLYLQMNSLRAEDTAVYYCAKDPGTTVIMSWFDPWGQGTLVTVSSASTKGPQVQLQESGPGLVKPSETLSLTCTVSGFSLIGYDLNWIRQPPGKGLEWIGIIWGDGTTDYNSAVKSRVTISKDTSKNQFSLKLSSVTAADTAVYYCARGGYWYATSYYFDYWGQGTLVTVSSASTKGPSVFPLAPCSRSTSESTAALGCLVKDYFPEPVTVSWNSGALTSGVHTFPAVLQSSGLYSLSSVVTVPSSSLGTKTYTCNVDHKPSNTKVDKRVESKYGPPCPPCPAPEFLGGPSVFLFPPKPKDTLMISRTPEVTCVVVDVSQEDPEVQFNWYVDGVEVHNAKTKPREEQFNSTYRVVSVLTVLHQDWLNGKEYKCKVSNKGLPSSIEKTISKAKGQPREPQVYTLPPSQEEMTKNQVSLTCLVKGFYPSDIAVEWESNGQPENNYKTTPPVLDSDGSFFLYSRLTVDKSRWQEGNVFSCSVMHEALHNHYTQKSLSLSLGK

SEQ ID NO: 101 - protein, 576 aa, Artificial sequence
  First chain of bispecific antibody 3
EVQLLESGGGLVQPGGSLRLSCAASGFTFSSYAMSWVRQAPGKGLEWVSGITGSGGSTYYADSVKGRFTISRDNSKNTLYLQMNSLRAEDTAVYYCVKDPGSTIIMSWFDPWGQGTLVTVSSASTKGPQVQLQESGPGLVKPSETLSLTCTVSGFSLIGYDLNWIRQPPGKGLEWIGIIWGDGTTDYNSAVKSRVTISKDTSKNQFSLKLSSVTAADTAVYYCARGGYWYATSYYFDYWGQGTLVTVSSASTKGPSVFPLAPCSRSTSESTAALGCLVKDYFPEPVTVSWNSGALTSGVHTFPAVLQSSGLYSLSSVVTVPSSSLGTKTYTCNVDHKPSNTKVDKRVESKYGPPCPPCPAPEFLGGPSVFLFPPKPKDTLMISRTPEVTCVVVDVSQEDPEVQFNWYVDGVEVHNAKTKPREEQFNSTYRVVSVLTVLHQDWLNGKEYKCKVSNKGLPSSIEKTISKAKGQPREPQVYTLPPSQEEMTKNQVSLTCLVKGFYPSDIAVEWESNGQPENNYKTTPPVLDSDGSFFLYSRLTVDKSRWQEGNVFSCSVMHEALHNHYTQKSLSLSLGK

SEQ ID NO: 102 - protein, 5 aa, Artificial sequence
  AMR2 HCDR1
DYDMS

SEQ ID NO: 103 - protein, 17 aa, Artificial sequence
  AMR2 HCDR2
WIYPSGGSIYYADSVKG

SEQ ID NO: 104 - protein, 18 aa, Artificial sequence
  AMR2 HCDR3
SGLTRTRWPIYYADGMDV

SEQ ID NO: 105 - protein, 13 aa, Artificial sequence
  AMR2 LCDR1
TGSSSNIGNNAVS

SEQ ID NO: 106 - protein, 7 aa, Artificial sequence
  AMR2 LCDR2
SDRHRPS

SEQ ID NO: 107 - protein, 11 aa, Artificial sequence
  AMR2 LCDR3
GSWDASLSGYV

SEQ ID NO: 108 - protein, 126 aa, Artificial sequence
  AMR2 heavy chain variable region
VQLLESGGGLVQPGGSLRLSCAASGFTFSDYDMSWVRQAPGKGLEWVSWIYPSGGSIYYADSVKGRFTISRDNSKNTLYLQMNSLRAEDTAVYYCARSGLTRTRWPIYYADGMDVWGQGTLVTVSS

SEQ ID NO: 109 - protein, 110 aa, Artificial sequence
  AMR2 light chain variable region
QSVLTQPPSASGTPGQRVTISCTGSSSNIGNNAVSWYQQLPGTAPKLLIYSDRHRPSGVPDRFSGSKSGTSASLAISGLRSEDEADYYCGSWDASLSGYVFGGGTKLTVL

SEQ ID NO: 110 - protein, 454 aa, Artificial sequence
  AMR2 heavy chain
EVQLLESGGGLVQPGGSLRLSCAASGFTFSDYDMSWVRQAPGKGLEWVSWIYPSGGSIYYADSVKGRFTISRDNSKNTLYLQMNSLRAEDTAVYYCARSGLTRTRWPIYYADGMDVWGQGTLVTVSSASTKGPSVFPLAPCSRSTSESTAALGCLVKDYFPEPVTVSWNSGALTSGVHTFPAVLQSSGLYSLSSVVTVPSSSLGTKTYTCNVDHKPSNTKVDKRVESKYGPPCPPCPAPEFLGGPSVFLFPPKPKDTLMISRTPEVTCVVVDVSQEDPEVQFNWYVDGVEVHNAKTKPREEQFNSTYRVVSVLTVLHQDWLNGKEYKCKVSNKGLPSSIEKTISKAKGQPREPQVYTLPPSQEEMTKNQVSLTCLVKGFYPSDIAVEWESNGQPENNYKTTPPVLDSDGSFFLYSRLTVDKSRWQEGNVFSCSVMHEALHNHYTQKSLSLSLGK

SEQ ID NO: 111 - protein, 216 aa, Artificial sequence
  AMR2 light chain
QSVLTQPPSASGTPGQRVTISCTGSSSNIGNNAVSWYQQLPGTAPKLLIYSDRHRPSGVPDRFSGSKSGTSASLAISGLRSEDEADYYCGSWDASLSGYVFGGGTKLTVLGQPKANPTVTLFPPSSEELQANKATLVCLISDFYPGAVTVAWKADGSPVKAGVETTKPSKQSNNKYAASSYLSLTPEQWKSHRSYSCQVTHEGSTVEKTVAPTECS